European Patent Application EP 4 218 418 A1, published August 2, 2023. Title: Anti-coccidial composition comprising mangosteen and uses thereof. Applicant: CJ CheilJedang Corporation. The sequence listing filed with the application follows.

SEQUENCE LISTING (4 sequences)

SEQ ID NO: 1 - DNA, 20 bp, Artificial Sequence
  synthetic_E.tenella ITS-1_Forward
tggaggggattatgagagga

SEQ ID NO: 2 - DNA, 20 bp, Artificial Sequence
  synthetic_E.tenella ITS-1_Reverse
caagcagcatgtaacggaga

SEQ ID NO: 3 - DNA, 22 bp, Artificial Sequence
  synthetic_E.acervulina ACE_Forward
gcagtccgatgaaaggtatttg

SEQ ID NO: 4 - DNA, 22 bp, Artificial Sequence
  synthetic_E.acervulina ACE_Reverse
gaagcgaaatgttaggccatct